European Patent Specification EP 3 571 305 B1, published May 22, 2024. Title: PLANT REGULATORY ELEMENTS AND USES THEREOF. Applicant: Monsanto Technology LLC. The sequence listing filed with the application follows.

SEQUENCE LISTING (57 sequences)

SEQ ID NO: 1 - DNA, 855 bp, Artificial
  Synthetic EXP, EXP-At.GSP442.nno+At.Cyco:3.
tgttaatgttatccgaactagtcataattacaaccgacaaaataaggttattttgtgtgttatagaattttttggacagtttttgttttggttttcgattgtagtaaaaatagatttatgtaataagatttacttttcttgttgaaacaaaataatcttagaattaactcaacttttatgttagaacaaatgataaaaaaatttccccttttctatgcgattattttcaatcagagagaaatacatataatatatataattcaaattaatctgccaaattaataaatttggattaaaatttataaatgaaacaatggtgtaaggcaattaaaaacacaacactaaaaatatgagaacattttatctgggcattaagagtttgggctttagatctaaaataaaggccggcccaacgagaatattaaaccctaattgacctagttccctatatatataaaccctatatttctctcgtcactcctcaactctcagctaaaccacggaccgcaggtaatttctctcctctctatttttaccattttccattgacgacgatctaggttttctgatttgattttggagaacgcctcgatgagtttatagattcgtagattggttttgagattcagtataatttcacccggattccaatttttgaaccgatacctaattttgaattgatttggtagatcgattggtcaaatttgaaattgatttttctccataatatctgaagcgtcttattggatcaaatctacaacatttctctgttgaaaggatcgattttttttttcttggaacatgataacttttgattattcatcaaagttttgttctttttaatatttcacaggt

SEQ ID NO: 2 - DNA, 480 bp, Artificial
  Synthetic promoter, P-At.GSP442.nno:2.
tgttaatgttatccgaactagtcataattacaaccgacaaaataaggttattttgtgtgttatagaattttttggacagtttttgttttggttttcgattgtagtaaaaatagatttatgtaataagatttacttttcttgttgaaacaaaataatcttagaattaactcaacttttatgttagaacaaatgataaaaaaatttccccttttctatgcgattattttcaatcagagagaaatacatataatatatataattcaaattaatctgccaaattaataaatttggattaaaatttataaatgaaacaatggtgtaaggcaattaaaaacacaacactaaaaatatgagaacattttatctgggcattaagagtttgggctttagatctaaaataaaggccggcccaacgagaatattaaaccctaattgacctagttccctatatatataaaccctatatttctctcgtcactc

SEQ ID NO: 3 - DNA, 20 bp, Artificial
  Synthetic leader, L-At.GSP442.nno:1.
ctcaactctcagctaaacca

SEQ ID NO: 4 - DNA, 500 bp, Artificial
  Synthetic EXP, EXP-At.GSP571.
agtacaatcatacaagagcaatatatatatttttggttattgaaatttaaatatcatcttcacaaaatgaaaaagcacaaaaagtattaattaatatcatgttttgagactcctttttaccaagaatataaatttcacacctaagaaaattctgaactaggaaaataaccagcatacaattaaggaataagaaaatgcaattacgataaacacttgtcacaaattgtttaataagtcactatccaatcaattatcaaaagtaagatattgccacgtggcaaccagtattttcatcaccttatcaaaagataagcaaaagaaccacatcaaagccacaaaatgccaaccacagatggataaggaaaatccaaccaaccacatgtaatcccacacctcatcaccttatccacacctctgtctatatatataaacacacacttcgtaaccactcatcactcaccacaaacagagaatatctcatctcttcttagcaaacaaag

SEQ ID NO: 5 - DNA, 500 bp, Artificial; identical to SEQ ID NO: 4
  Synthetic promoter, P-At.GSP571.nno:5.

SEQ ID NO: 6 - DNA, 49 bp, Artificial
  Synthetic leader, L-At.GSP571.nno:1.
atcactcaccacaaacagagaatatctcatctcttcttagcaaacaaag

SEQ ID NO: 7 - DNA, 855 bp, Artificial
  Synthetic EXP, EXP-At.GSP571.nno+At.Cyco:2.
agtacaatcatacaagagcaatatatatatttttggttattgaaatttaaatatcatcttcacaaaatgaaaaagcacaaaaagtattaattaatatcatgttttgagactcctttttaccaagaatataaatttcacacctaagaaaattctgaactaggaaaataaccagcatacaattaaggaataagaaaatgcaattacgataaacacttgtcacaaattgtttaataagtcactatccaatcaattatcaaaagtaagatattgccacgtggcaaccagtattttcatcaccttatcaaaagataagcaaaagaaccacatcaaagccacaaaatgccaaccacagatggataaggaaaatccaaccaaccacatgtaatcccacacctcatcaccttatccacacctctgtctatatatataaacacacacttcgtaaccactcatcactcaccacaaacagagaatatctcatctcttcttagcaaacaaagcggaccgcaggtaatttctctcctctctatttttaccattttccattgacgacgatctaggttttctgatttgattttggagaacgcctcgatgagtttatagattcgtagattggttttgagattcagtataatttcacccggattccaatttttgaaccgatacctaattttgaattgatttggtagatcgattggtcaaatttgaaattgatttttctccataatatctgaagcgtcttattggatcaaatctacaacatttctctgttgaaaggatcgattttttttttcttggaacatgataacttttgattattcatcaaagttttgttctttttaatatttcacaggt

SEQ ID NO: 8 - DNA, 816 bp, Artificial
  Synthetic EXP, EXP-At.GSP571.nno+At.GSI21.nno:10.
agtacaatcatacaagagcaatatatatatttttggttattgaaatttaaatatcatcttcacaaaatgaaaaagcacaaaaagtattaattaatatcatgttttgagactcctttttaccaagaatataaatttcacacctaagaaaattctgaactaggaaaataaccagcatacaattaaggaataagaaaatgcaattacgataaacacttgtcacaaattgtttaataagtcactatccaatcaattatcaaaagtaagatattgccacgtggcaaccagtattttcatcaccttatcaaaagataagcaaaagaaccacatcaaagccacaaaatgccaaccacagatggataaggaaaatccaaccaaccacatgtaatcccacacctcatcaccttatccacacctctgtctatatatataaacacacacttcgtaaccactcatcactcaccacaaacagagaatatctcatctcttcttagcaaacaaagcggaccgcaggtttattcttctctctctatcctctctcttctgatctcgatttgtttttttcgaatcgctctacttccagttagattcttgatttgagattaattagattgattattctaatcgttttttttgtaagcaattaagatttatcttgttttatgtttttctttaggtatgacttgttatgtatgtcactgtttcagatctgatcctctctgttggtttgtgaattctcttgtattgttctaatcactgtttctgaatttgattcgggtttttattgaattctttttatgtgttttggtatttgcaggt

SEQ ID NO: 9 - DNA, 309 bp, Artificial
  Synthetic intron, I-At.GSI21.nno:2.
caggtttattcttctctctctatcctctctcttctgatctcgatttgtttttttcgaatcgctctacttccagttagattcttgatttgagattaattagattgattattctaatcgttttttttgtaagcaattaagatttatcttgttttatgtttttctttaggtatgacttgttatgtatgtcactgtttcagatctgatcctctctgttggtttgtgaattctcttgtattgttctaatcactgtttctgaatttgattcgggtttttattgaattctttttatgtgttttggtatttgcaggt

SEQ ID NO: 10 - DNA, 810 bp, Artificial
  Synthetic EXP, EXP-At.GSP571.nno+At.GSI102.nno:1.
agtacaatcatacaagagcaatatatatatttttggttattgaaatttaaatatcatcttcacaaaatgaaaaagcacaaaaagtattaattaatatcatgttttgagactcctttttaccaagaatataaatttcacacctaagaaaattctgaactaggaaaataaccagcatacaattaaggaataagaaaatgcaattacgataaacacttgtcacaaattgtttaataagtcactatccaatcaattatcaaaagtaagatattgccacgtggcaaccagtattttcatcaccttatcaaaagataagcaaaagaaccacatcaaagccacaaaatgccaaccacagatggataaggaaaatccaaccaaccacatgtaatcccacacctcatcaccttatccacacctctgtctatatatataaacacacacttcgtaaccactcatcactcaccacaaacagagaatatctcatctcttcttagcaaacaaagtttcaggtttagctttctctccgatctcggctttcgatctgatctcgtctgatctccgatttcgatccccgtccgatctcgatctgatcccatccgatctgtgattgattcgttgagattcagatctgatcttaggatctctctgatagatcatagattcaatctctcgagatagagatgattgatgttgttcagatcggttttgatctctgatctgatcagctcgattgattcgatttgattctcgattcgatttgatcgacaattgatctgattctctaattgatgttctgtttttgttacaggtttt

SEQ ID NO: 11 - DNA, 310 bp, Artificial
  Synthetic intron, I-At.GSI102.nno:1.
tttcaggtttagctttctctccgatctcggctttcgatctgatctcgtctgatctccgatttcgatccccgtccgatctcgatctgatcccatccgatctgtgattgattcgttgagattcagatctgatcttaggatctctctgatagatcatagattcaatctctcgagatagagatgattgatgttgttcagatcggttttgatctctgatctgatcagctcgattgattcgatttgattctcgattcgatttgatcgacaattgatctgattctctaattgatgttctgtttttgttacaggtttt

SEQ ID NO: 12 - DNA, 500 bp, Artificial
  Synthetic EXP, EXP-At.GSP564.
agagttacaatatagagaaaaaatgtattctgtgtttttcacttttcttcttctttgaaaatccaaaaacaactatttattgattggcaaattgcatcaaatttttcatgctaaatccaacataaatataaaatcttttaatcaaatacagaatctaaagatagtagggttttttttatttaaaatgatgtttcaaaaaattagaaagcatgttttccacacttggaaaatataaataaattaagatttattttttcccaaacaagataaatctataaatattcatcacaatcacgtgtacaaaaataaatccaacaagagataaggataagccaacggacccatatattaggcccattttaaaataaggaaataagcagataattatccaccaccttatccaaaaccctagatccacaacataaatctctataaaaacccttttcactcacactcacatcactcacataagaactaaaatctctaaagagtcgtctctg

SEQ ID NO: 13 - DNA, 461 bp, Artificial
  Synthetic promoter, P-At.GSP564.nno:3.
agagttacaatatagagaaaaaatgtattctgtgtttttcacttttcttcttctttgaaaatccaaaaacaactatttattgattggcaaattgcatcaaatttttcatgctaaatccaacataaatataaaatcttttaatcaaatacagaatctaaagatagtagggttttttttatttaaaatgatgtttcaaaaaattagaaagcatgttttccacacttggaaaatataaataaattaagatttattttttcccaaacaagataaatctataaatattcatcacaatcacgtgtacaaaaataaatccaacaagagataaggataagccaacggacccatatattaggcccattttaaaataaggaaataagcagataattatccaccaccttatccaaaaccctagatccacaacataaatctctataaaaacccttttcactcacactcacatc

SEQ ID NO: 14 - DNA, 39 bp, Artificial
  Synthetic leader, L-At.GSP564.nno:1.
actcacataagaactaaaatctctaaagagtcgtctctg

SEQ ID NO: 15 - DNA, 855 bp, Artificial
  Synthetic EXP, EXP-At.GSP564.nno+At.Cyco:2.
agagttacaatatagagaaaaaatgtattctgtgtttttcacttttcttcttctttgaaaatccaaaaacaactatttattgattggcaaattgcatcaaatttttcatgctaaatccaacataaatataaaatcttttaatcaaatacagaatctaaagatagtagggttttttttatttaaaatgatgtttcaaaaaattagaaagcatgttttccacacttggaaaatataaataaattaagatttattttttcccaaacaagataaatctataaatattcatcacaatcacgtgtacaaaaataaatccaacaagagataaggataagccaacggacccatatattaggcccattttaaaataaggaaataagcagataattatccaccaccttatccaaaaccctagatccacaacataaatctctataaaaacccttttcactcacactcacatcactcacataagaactaaaatctctaaagagtcgtctctgcggaccgcaggtaatttctctcctctctatttttaccattttccattgacgacgatctaggttttctgatttgattttggagaacgcctcgatgagtttatagattcgtagattggttttgagattcagtataatttcacccggattccaatttttgaaccgatacctaattttgaattgatttggtagatcgattggtcaaatttgaaattgatttttctccataatatctgaagcgtcttattggatcaaatctacaacatttctctgttgaaaggatcgattttttttttcttggaacatgataacttttgattattcatcaaagttttgttctttttaatatttcacaggt

SEQ ID NO: 16 - DNA, 807 bp, Artificial
  Synthetic EXP, EXP-At.GSP564.nno+At.GSI17.nno:2.
agagttacaatatagagaaaaaatgtattctgtgtttttcacttttcttcttctttgaaaatccaaaaacaactatttattgattggcaaattgcatcaaatttttcatgctaaatccaacataaatataaaatcttttaatcaaatacagaatctaaagatagtagggttttttttatttaaaatgatgtttcaaaaaattagaaagcatgttttccacacttggaaaatataaataaattaagatttattttttcccaaacaagataaatctataaatattcatcacaatcacgtgtacaaaaataaatccaacaagagataaggataagccaacggacccatatattaggcccattttaaaataaggaaataagcagataattatccaccaccttatccaaaaccctagatccacaacataaatctctataaaaacccttttcactcacactcacatcactcacataagaactaaaatctctaaagagtcgtctctgcggaccgcaggtaaacccagatctctttcttctcttctcttcatctcgatctctccattttcataaacccaattttttctctgatttgtttgatttggtttggatctttctgtgtttccatggttttaggaattttaggatagatttttgtttgttcatgttattcatcggatatatagatttcaaattcttttgcaatttttctctctctttagttttgctcaattttggttgttgttgtgatgagtgttctctttatgggtttatctgagcttggtgagagttttttgatattgattttgcaggt

SEQ ID NO: 17 - DNA, 300 bp, Artificial
  Synthetic intron, I-At.GSI17.nno:1.
caggtaaacccagatctctttcttctcttctcttcatctcgatctctccattttcataaacccaattttttctctgatttgtttgatttggtttggatctttctgtgtttccatggttttaggaattttaggatagatttttgtttgttcatgttattcatcggatatatagatttcaaattcttttgcaatttttctctctctttagttttgctcaattttggttgttgttgtgatgagtgttctctttatgggtttatctgagcttggtgagagttttttgatattgattttgcaggt

SEQ ID NO: 18 - DNA, 810 bp, Artificial
  Synthetic EXP, EXP-At.GSP564.nno+At.GSI102.nno:1.
agagttacaatatagagaaaaaatgtattctgtgtttttcacttttcttcttctttgaaaatccaaaaacaactatttattgattggcaaattgcatcaaatttttcatgctaaatccaacataaatataaaatcttttaatcaaatacagaatctaaagatagtagggttttttttatttaaaatgatgtttcaaaaaattagaaagcatgttttccacacttggaaaatataaataaattaagatttattttttcccaaacaagataaatctataaatattcatcacaatcacgtgtacaaaaataaatccaacaagagataaggataagccaacggacccatatattaggcccattttaaaataaggaaataagcagataattatccaccaccttatccaaaaccctagatccacaacataaatctctataaaaacccttttcactcacactcacatcactcacataagaactaaaatctctaaagagtcgtctctgtttcaggtttagctttctctccgatctcggctttcgatctgatctcgtctgatctccgatttcgatccccgtccgatctcgatctgatcccatccgatctgtgattgattcgttgagattcagatctgatcttaggatctctctgatagatcatagattcaatctctcgagatagagatgattgatgttgttcagatcggttttgatctctgatctgatcagctcgattgattcgatttgattctcgattcgatttgatcgacaattgatctgattctctaattgatgttctgtttttgttacaggtttt

SEQ ID NO: 19 - DNA, 500 bp, Artificial
  Synthetic EXP, EXP-At.GSP579.
catagagcagtcttgtctcaaaaaaatcgaattaagcagttgaaagtgttcgtcttatcaagatgaaaatctgacaaaaattttgttaaaatttggtagtatttgataagatatgtaccttaaaattgatgttaataatcttcttatccaaaaaaagaaccaatccattgcagtcttaaatgaaatatttcaagaaaggattgagccaaaaaccgtgtttataaaattttcaaatccacaatttccacattcacttggatattacaagtgtggcatctcataaaaaaaaagaaaaagaaaaaccacgtggactattatatccagccacgtggctttaaaatcttatccaaaatcacctctcatccaacggataaggtaaccacacagccttatccaaccacatcacacgaatccactctatatatactccatataaccatcactcacacgtctttcatcacacaagtaaaacagcatcactaaaagaaaaaaaacaagaa

SEQ ID NO: 20 - DNA, 449 bp, Artificial
  Synthetic promoter, P-At.GSP579.nno:2.
catagagcagtcttgtctcaaaaaaatcgaattaagcagttgaaagtgttcgtcttatcaagatgaaaatctgacaaaaattttgttaaaatttggtagtatttgataagatatgtaccttaaaattgatgttaataatcttcttatccaaaaaaagaaccaatccattgcagtcttaaatgaaatatttcaagaaaggattgagccaaaaaccgtgtttataaaattttcaaatccacaatttccacattcacttggatattacaagtgtggcatctcataaaaaaaaagaaaaagaaaaaccacgtggactattatatccagccacgtggctttaaaatcttatccaaaatcacctctcatccaacggataaggtaaccacacagccttatccaaccacatcacacgaatccactctatatatactccatataaccatcactcacac

SEQ ID NO: 21 - DNA, 51 bp, Artificial
  Synthetic leader, L-At.GSP579.nno:1.
gtctttcatcacacaagtaaaacagcatcactaaaagaaaaaaaacaagaa

SEQ ID NO: 22 - DNA, 810 bp, Artificial
  Synthetic EXP, EXP-At.GSP579.nno+At.GSI102.nno:3.
catagagcagtcttgtctcaaaaaaatcgaattaagcagttgaaagtgttcgtcttatcaagatgaaaatctgacaaaaattttgttaaaatttggtagtatttgataagatatgtaccttaaaattgatgttaataatcttcttatccaaaaaaagaaccaatccattgcagtcttaaatgaaatatttcaagaaaggattgagccaaaaaccgtgtttataaaattttcaaatccacaatttccacattcacttggatattacaagtgtggcatctcataaaaaaaaagaaaaagaaaaaccacgtggactattatatccagccacgtggctttaaaatcttatccaaaatcacctctcatccaacggataaggtaaccacacagccttatccaaccacatcacacgaatccactctatatatactccatataaccatcactcacacgtctttcatcacacaagtaaaacagcatcactaaaagaaaaaaaacaagaatttcaggtttagctttctctccgatctcggctttcgatctgatctcgtctgatctccgatttcgatccccgtccgatctcgatctgatcccatccgatctgtgattgattcgttgagattcagatctgatcttaggatctctctgatagatcatagattcaatctctcgagatagagatgattgatgttgttcagatcggttttgatctctgatctgatcagctcgattgattcgatttgattctcgattcgatttgatcgacaattgatctgattctctaattgatgttctgtttttgttacaggtttt

SEQ ID NO: 23 - DNA, 1350 bp, Artificial
  Synthetic EXP, EXP-At.GSP571.nno+At.GSP442.nno+At.Cyco:1.
agtacaatcatacaagagcaatatatatatttttggttattgaaatttaaatatcatcttcacaaaatgaaaaagcacaaaaagtattaattaatatcatgttttgagactcctttttaccaagaatataaatttcacacctaagaaaattctgaactaggaaaataaccagcatacaattaaggaataagaaaatgcaattacgataaacacttgtcacaaattgtttaataagtcactatccaatcaattatcaaaagtaagatattgccacgtggcaaccagtattttcatcaccttatcaaaagataagcaaaagaaccacatcaaagccacaaaatgccaaccacagatggataaggaaaatccaaccaaccacatgtaatcccacacctcatcaccttatccacacctctgtctattgttaatgttatccgaactagtcataattacaaccgacaaaataaggttattttgtgtgttatagaattttttggacagtttttgttttggttttcgattgtagtaaaaatagatttatgtaataagatttacttttcttgttgaaacaaaataatcttagaattaactcaacttttatgttagaacaaatgataaaaaaatttccccttttctatgcgattattttcaatcagagagaaatacatataatatatataattcaaattaatctgccaaattaataaatttggattaaaatttataaatgaaacaatggtgtaaggcaattaaaaacacaacactaaaaatatgagaacattttatctgggcattaagagtttgggctttagatctaaaataaaggccggcccaacgagaatattaaaccctaattgacctagttccctatatatataaaccctatatttctctcgtcactcctcaactctcagctaaaccacggaccgcagtgagtcacataaccctcttggaaagagtctcaacacttgcagagaaaaagaacaaggaagatcccggaaacaggtaatttctctcctctctatttttaccattttccattgacgacgatctaggttttctgatttgattttggagaacgcctcgatgagtttatagattcgtagattggttttgagattcagtataatttcacccggattccaatttttgaaccgatacctaattttgaattgatttggtagatcgattggtcaaatttgaaattgatttttctccataatatctgaagcgtcttattggatcaaatctacaacatttctctgttgaaaggatcgattttttttttcttggaacatgataacttttgattattcatcaaagttttgttctttttaatatttcacaggt

SEQ ID NO: 24 - DNA, 422 bp, Artificial
  Synthetic enhancer, E-At.GSP571.nno:1.
agtacaatcatacaagagcaatatatatatttttggttattgaaatttaaatatcatcttcacaaaatgaaaaagcacaaaaagtattaattaatatcatgttttgagactcctttttaccaagaatataaatttcacacctaagaaaattctgaactaggaaaataaccagcatacaattaaggaataagaaaatgcaattacgataaacacttgtcacaaattgtttaataagtcactatccaatcaattatcaaaagtaagatattgccacgtggcaaccagtattttcatcaccttatcaaaagataagcaaaagaaccacatcaaagccacaaaatgccaaccacagatggataaggaaaatccaaccaaccacatgtaatcccacacctcatcaccttatccacacctctgtctat

SEQ ID NO: 25 - DNA, 902 bp, Artificial
  Synthetic chimeric promoter, P-At.GSP571/442.
agtacaatcatacaagagcaatatatatatttttggttattgaaatttaaatatcatcttcacaaaatgaaaaagcacaaaaagtattaattaatatcatgttttgagactcctttttaccaagaatataaatttcacacctaagaaaattctgaactaggaaaataaccagcatacaattaaggaataagaaaatgcaattacgataaacacttgtcacaaattgtttaataagtcactatccaatcaattatcaaaagtaagatattgccacgtggcaaccagtattttcatcaccttatcaaaagataagcaaaagaaccacatcaaagccacaaaatgccaaccacagatggataaggaaaatccaaccaaccacatgtaatcccacacctcatcaccttatccacacctctgtctattgttaatgttatccgaactagtcataattacaaccgacaaaataaggttattttgtgtgttatagaattttttggacagtttttgttttggttttcgattgtagtaaaaatagatttatgtaataagatttacttttcttgttgaaacaaaataatcttagaattaactcaacttttatgttagaacaaatgataaaaaaatttccccttttctatgcgattattttcaatcagagagaaatacatataatatatataattcaaattaatctgccaaattaataaatttggattaaaatttataaatgaaacaatggtgtaaggcaattaaaaacacaacactaaaaatatgagaacattttatctgggcattaagagtttgggctttagatctaaaataaaggccggcccaacgagaatattaaaccctaattgacctagttccctatatatataaaccctatatttctctcgtcactc

SEQ ID NO: 26 - DNA, 800 bp, Artificial
  Synthetic EXP, EXP-At.GSP576.nno+At.GSI17.nno:3.
aattaaattcaacacgtttgttatatattttttattgaaattattcttcattcgtcttttaatggataaaaaggtataatcaagtatattttatacacatctttctatttgtgtgtaccaaatgttaaaatggccaattttgaccaaaaaaccgcataattttcttaatttcttaaatatgattaattcatcaataacttggaatttcacaatacacaaaagtgggtgtagttaccgttattatatttatacacaacaactcatctcctcatagaaagaaaagaaaaataaaataagaaatcaaaaaacgacaagataaccaatctccacatcatccacgtggcgtaaggataaggtcacaaccaccactcagccacgtggcagaatcttatccaatcactctcaccacacaaaccttatccacttctatatataatctcttcttctcattatcactcaccacacatccttgcaaaagtaaagagaaaaaacaaacaagacaggtaaacccagatctctttcttctcttctcttcatctcgatctctccattttcataaacccaattttttctctgatttgtttgatttggtttggatctttctgtgtttccatggttttaggaattttaggatagatttttgtttgttcatgttattcatcggatatatagatttcaaattcttttgcaatttttctctctctttagttttgctcaattttggttgttgttgtgatgagtgttctctttatgggtttatctgagcttggtgagagttttttgatattgattttgcaggt

SEQ ID NO: 27 - DNA, 458 bp, Artificial
  Synthetic promoter, P-At.GSP576.nno:4.
aattaaattcaacacgtttgttatatattttttattgaaattattcttcattcgtcttttaatggataaaaaggtataatcaagtatattttatacacatctttctatttgtgtgtaccaaatgttaaaatggccaattttgaccaaaaaaccgcataattttcttaatttcttaaatatgattaattcatcaataacttggaatttcacaatacacaaaagtgggtgtagttaccgttattatatttatacacaacaactcatctcctcatagaaagaaaagaaaaataaaataagaaatcaaaaaacgacaagataaccaatctccacatcatccacgtggcgtaaggataaggtcacaaccaccactcagccacgtggcagaatcttatccaatcactctcaccacacaaaccttatccacttctatatataatctcttcttctcattatcactc

SEQ ID NO: 28 - DNA, 42 bp, Artificial
  Synthetic leader, L-At.GSP576.nno:2.
accacacatccttgcaaaagtaaagagaaaaaacaaacaaga

SEQ ID NO: 29 - DNA, 400 bp, Artificial
  Synthetic 3' UTR, T-Zm.GST59.nno:1.
ttgttttgtttgtaccataatatatttgctgtgtgtttgctgccatctcatgtgcagaggaatatatattttttcgtggtttctgtcgtgctgtactgaggaccgttgtaaacatatgaataaaagtaataaatttgttttttgtttcataccccattggtggtgctcctttggttctcgtttgttgctggagacagatatgtttgtgttgtttgtgttcttgttttatctggaggcgagcagctttttgtttgggaagaacaaaatcagtttggatgctttgctccatcctgtactgttgtaaactgcatatatatatatatatatgaataaaactggttttgtttcataccatgtttgtgtgttctgttctgttgctcgagacgaggaataaattgtt

SEQ ID NO: 30 - DNA, 947 bp, Artificial
  Synthetic EXP, EXP-At.GSP221+At.Cyco:3.
gctagcgcttatggagcgtgatggactgaaagagacccctaccacgtgttgacgtaagcaatgacataaaaccgatcctaatctctcctacgaacgacagcggagagtactgctgaaagctatgcttttatttttctttatttttctcgtcagtggaatacacgttttgtcggtgtgtgtccttttccaaagaaagacggaactgcctaggacaacgtcggctaccaaagcacaatgtaaagtagacatgatgatcgacgacgtcatgcatgacgtttaacatgcattgtatgtgtccgtcagtctataaataggtcaagaacaaacatcgagaaaaggcagaggcgaaatacccatctgcctatctctcaagaaataactctctcttgttcttcatcctttctttcatagtttaaaaacctgaaattgggcaagccccataggcattttggtatcagagcgagtaaggacaagtaggtaagtccctaaaatacttctatcaataaaatttctacgccaagaagggtaagttgtacgtttatcctacacccttgtgtttgtaaccaggcttggtcaagtgcacaagggtatttgagtcccaggtaatttctctcctctctatttttaccattttccattgacgacgatctaggttttctgatttgattttggagaacgcctcgatgagtttatagattcgtagattggttttgagattcagtataatttcacccggattccaatttttgaaccgatacctaattttgaattgatttggtagatcgattggtcaaatttgaaattgatttttctccataatatctgaagcgtcttattggatcaaatctacaacatttctctgttgaaaggatcgattttttttttcttggaacatgataacttttgattattcatcaaagttttgttctttttaatatttcacaggt

SEQ ID NO: 31 - DNA, 370 bp, Artificial
  Synthetic promoter, P-At.GSP221:3.
gctagcgcttatggagcgtgatggactgaaagagacccctaccacgtgttgacgtaagcaatgacataaaaccgatcctaatctctcctacgaacgacagcggagagtactgctgaaagctatgcttttatttttctttatttttctcgtcagtggaatacacgttttgtcggtgtgtgtccttttccaaagaaagacggaactgcctaggacaacgtcggctaccaaagcacaatgtaaagtagacatgatgatcgacgacgtcatgcatgacgtttaacatgcattgtatgtgtccgtcagtctataaataggtcaagaacaaacatcgagaaaaggcagaggcgaaatacccatctgcctatctctc

SEQ ID NO: 32 - DNA, 229 bp, Artificial
  Synthetic leader, L-At.GSP221:1.
aagaaataactctctcttgttcttcatcctttctttcatagtttaaaaacctgaaattgggcaagccccataggcattttggtatcagagcgagtaaggacaagtaggtaagtccctaaaatacttctatcaataaaatttctacgccaagaagggtaagttgtacgtttatcctacacccttgtgtttgtaaccaggcttggtcaagtgcacaagggtatttgagtcc

SEQ ID NO: 33 - DNA, 348 bp, Arabidopsis thaliana
  misc_feature (1)..(348): An intron, I-At.Cyco:2 derived from a Cytochrome c oxidase subunit VIa gene from Arabidopsis.
caggtaatttctctcctctctatttttaccattttccattgacgacgatctaggttttctgatttgattttggagaacgcctcgatgagtttatagattcgtagattggttttgagattcagtataatttcacccggattccaatttttgaaccgatacctaattttgaattgatttggtagatcgattggtcaaatttgaaattgatttttctccataatatctgaagcgtcttattggatcaaatctacaacatttctctgttgaaaggatcgattttttttttcttggaacatgataacttttgattattcatcaaagttttgttctttttaatatttcacaggt

SEQ ID NO: 34 - DNA, 500 bp, Medicago truncatula
  misc_feature (1)..(500): 3' UTR, T-Mt.Sali3-2-1:2:1 derived from the Sali3 gene of Medicago truncatula.
gagtactctccaacatggacacaccatgggattgtgtaacataaataatgtgtcgtttgtaatgaatgctcgcaacttttctagctaattaagctagagttgaacttgagctacttttatgtaccctaaagaggcacaatctttgctgttgatgtactatgatcatgttataatatgatgaaaatggagtgtgcctcattttataatttttattttcctgagtatatgtttttagggctaaacaccttataaaaaaaggtcacttagaatatgaaacatgaacttttgtaaaaaagtagagattaaaattgaaatcaaaaatttttataggatcaatattcgaagaatttttttagagggattaaaattaaatatagtttcggactgacccaaggcacaatccggctccgctcgggttcgacctgagtccaccatgcatctgtcaccttaccattgacacgccctaaaatacattagatcgcagtacaaattgagagtta

SEQ ID NO: 35 - DNA, 500 bp, Medicago truncatula
  misc_feature (1)..(500): 3' UTR, T-Mt.Oxr-1:2:1 derived from a putative oxidoreductase (OXR) protein gene from Medicago truncatula.
aaatgaatgaatcagctttctcttgttcataaagaattgtgtggaaatgaattgtgtgttgctatatacatgagtgtgttggttgctgccttatgtgttcttctagggttattttttcttttgctttgtaataatttgtgcgttactattgtaaacaatgtatttaatgaataatgaaagtctaaagtttgtaatggagggaagtaaatgtaaatcctttcgcaagtgtttttttagcttgaaagtctttcatgcattggtttggagtaccatcatatcacccttaatttttctagttatgattttagggacaagagaagttcaaattacactccaattatgtgctcggggaaatttaattggtagcagacaatacacgaaaaagtaacacatttagtatcttactatcatctgcaaatcgtgcatatgttcatatcatttcacatttttataatccagcatattataaattcaaacctaattttggtacataatagtat

SEQ ID NO: 36 - DNA, 315 bp, Gossypium barbadense
  misc_feature (1)..(315): 3' UTR, T-Gb.FbL2:1 derived from the Gossypium barbadense FbLate-2 gene.
accatatgacactggtgcatgtgccatcatcatgcagtaatttcatggtatatcttaattatatggttaataaaaaaaagatggtgagtgaataatgtgcgtgcattcctccatgcaccaatggtgaatctctttgcatacatagagattctgaatgattatagtttatgttgtagtgaaattaattttgaatgttgtttttaaattttaatgtcacttggcttgatttatgttttaacgaagcttatgttatgtattttactttaatgatattgcatgtattgttaatttaacattgcttgatcagtatactct

SEQ ID NO: 37 - DNA, 500 bp, Medicago truncatula
  misc_feature (1)..(500): 3' UTR, T-Mt.RD22-1:2:1 derived from a dehydration-responsive protein RD22 gene from Medicago truncatula.
aaacaccaattccatcttcttcaataataaccactatatatatatagaagcaacttcaaaaatacttaatacttgtattataaattgagttactttgaatgtcctacgatagagacggagttcaaatctcctcaagtatggttgaaaaatggtcttcaatgtaactttaaataaaaactttgtacgtcctcgctaataaaaataatgtttgtttaattactttatatatgtattttttaatgctattttatatatgttgtaccccaaacttgtctgaccaatttaatcagaagaacatgtagagtgtaggtttgccgggaagatttggattaaagtcttcgtttggttgggtttggtcttggtcatgccggaaaatttattttccttgtacttcaaatgttttgctttttcgatcggaaagggaataggagattaaagggcctccttttaatatggcaaacagaattatagctttagactgacgctgcggtttagcttca

SEQ ID NO: 38 - DNA, 1204 bp, Arabidopsis thaliana
  misc_feature (1)..(1204): EXP-At.Cyco:1:1, derived from a Cytochrome c oxidase subunit VIa gene from Arabidopsis.
tgcgagtgggcgaattccggagcactctgattggctgaaaaaatagaaatagtagtgatgttgctcctcctctcctcctctattattaatttttcgtcgttcttcttctgaaagttgtgtggtttttagaggtcaccaaaaaaaatctattttgagatactaaaaatatttcgttttgcattttgttgtgcagccatttgttacacaggttgaagcttataactgaaaattggattcaaagaatcgtagatgaagaaatcgaagtgagttgaatattttctgaacatatgaaaattggaacaagttttttctcattttgctagtttcctgtttttatgttttcttgactttaggagatgacatatggaggtgaactatacaaaggttgttgcaacgataacattctccttaattcagtttttgcaactcggttacaagcactcagtggacttttggccaagacaattttttttttttttttctctctctctaaaatgttatagatacgaatcctttgttgaataaaggaaaaagttgaacatttgattacacataagactttaacataatccaacttttttttatatgaagctacaaacaagatttaaaacatcaaagattccatctaaacttcattcatcttcaatcttcaacatccttcaatgactagtatgtatgtacataagtaaaattgttgataagaaaacaaaacaatgatgggctaaaatagcccataaaaggcccattaaacttgggtttagactttagattcaacgacgccagattagtgagtcacataaccctcttggaaagagtctcaacacttgcagagaaaaagaacaaggaagatcccggaaacaggtaatttctctcctctctatttttaccattttccattgacgacgatctaggttttctgatttgattttggagaacgcctcgatgagtttatagattcgtagattggttttgagattcagtataatttcacccggattccaatttttgaaccgatacctaattttgaattgatttggtagatcgattggtcaaatttgaaattgatttttctccataatatctgaagcgtcttattggatcaaatctacaacatttctctgttgaaaggatcgattttttttttcttggaacatgataacttttgattattcatcaaagttttgttctttttaatatttcacag

SEQ ID NO: 39 - DNA, 786 bp, Arabidopsis thaliana
  misc_feature (1)..(786): Promoter, P-At.Cyco-1:1:2 derived from a Cytochrome c oxidase subunit VIa gene from Arabidopsis.
tgcgagtgggcgaattccggagcactctgattggctgaaaaaatagaaatagtagtgatgttgctcctcctctcctcctctattattaatttttcgtcgttcttcttctgaaagttgtgtggtttttagaggtcaccaaaaaaaatctattttgagatactaaaaatatttcgttttgcattttgttgtgcagccatttgttacacaggttgaagcttataactgaaaattggattcaaagaatcgtagatgaagaaatcgaagtgagttgaatattttctgaacatatgaaaattggaacaagttttttctcattttgctagtttcctgtttttatgttttcttgactttaggagatgacatatggaggtgaactatacaaaggttgttgcaacgataacattctccttaattcagtttttgcaactcggttacaagcactcagtggacttttggccaagacaattttttttttttttttctctctctctaaaatgttatagatacgaatcctttgttgaataaaggaaaaagttgaacatttgattacacataagactttaacataatccaacttttttttatatgaagctacaaacaagatttaaaacatcaaagattccatctaaacttcattcatcttcaatcttcaacatccttcaatgactagtatgtatgtacataagtaaaattgttgataagaaaacaaaacaatgatgggctaaaatagcccataaaaggcccattaaacttgggtttagactttagattcaacgacgccagatt

SEQ ID NO: 40 - DNA, 72 bp, Arabidopsis thaliana
  misc_feature (1)..(72): Leader, L-At.Cyco-1:1:2 derived from a Cytochrome c oxidase subunit VIa gene from Arabidopsis.
agtgagtcacataaccctcttggaaagagtctcaacacttgcagagaaaaagaacaaggaagatcccggaaa

SEQ ID NO: 41 - DNA, 346 bp, Arabidopsis thaliana
  misc_feature (1)..(346): Intron, I-At.Cyco-1:1:1 derived from a Cytochrome c oxidase subunit VIa gene from Arabidopsis.
caggtaatttctctcctctctatttttaccattttccattgacgacgatctaggttttctgatttgattttggagaacgcctcgatgagtttatagattcgtagattggttttgagattcagtataatttcacccggattccaatttttgaaccgatacctaattttgaattgatttggtagatcgattggtcaaatttgaaattgatttttctccataatatctgaagcgtcttattggatcaaatctacaacatttctctgttgaaaggatcgattttttttttcttggaacatgataacttttgattattcatcaaagttttgttctttttaatatttcacag

SEQ ID NO: 42 - DNA, 2001 bp, Artificial
  Coding sequence for beta-glucuronidase (GUS) with a processable intron derived from the potato light-inducible tissue-specific ST-LS1 gene (Genbank Accession: X04753).
atggtccgtcctgtagaaaccccaacccgtgaaatcaaaaaactcgacggcctgtgggcattcagtctggatcgcgaaaactgtggaattgatcagcgttggtgggaaagcgcgttacaagaaagccgggcaattgctgtgccaggcagttttaacgatcagttcgccgatgcagatattcgtaattatgcgggcaacgtctggtatcagcgcgaagtctttataccgaaaggttgggcaggccagcgtatcgtgctgcgtttcgatgcggtcactcattacggcaaagtgtgggtcaataatcaggaagtgatggagcatcagggcggctatacgccatttgaagccgatgtcacgccgtatgttattgccgggaaaagtgtacgtaagtttctgcttctacctttgatatatatataataattatcattaattagtagtaatataatatttcaaatatttttttcaaaataaaagaatgtagtatatagcaattgcttttctgtagtttataagtgtgtatattttaatttataacttttctaatatatgaccaaaatttgttgatgtgcaggtatcaccgtttgtgtgaacaacgaactgaactggcagactatcccgccgggaatggtgattaccgacgaaaacggcaagaaaaagcagtcttacttccatgatttctttaactatgccggaatccatcgcagcgtaatgctctacaccacgccgaacacctgggtggacgatatcaccgtggtgacgcatgtcgcgcaagactgtaaccacgcgtctgttgactggcaggtggtggccaatggtgatgtcagcgttgaactgcgtgatgcggatcaacaggtggttgcaactggacaaggcactagcgggactttgcaagtggtgaatccgcacctctggcaaccgggtgaaggttatctctatgaactgtgcgtcacagccaaaagccagacagagtgtgatatctacccgcttcgcgtcggcatccggtcagtggcagtgaagggcgaacagttcctgattaaccacaaaccgttctactttactggctttggtcgtcatgaagatgcggacttgcgtggcaaaggattcgataacgtgctgatggtgcacgaccacgcattaatggactggattggggccaactcctaccgtacctcgcattacccttacgctgaagagatgctcgactgggcagatgaacatggcatcgtggtgattgatgaaactgctgctgtcggctttaacctctctttaggcattggtttcgaagcgggcaacaagccgaaagaactgtacagcgaagaggcagtcaacggggaaactcagcaagcgcacttacaggcgattaaagagctgatagcgcgtgacaaaaaccacccaagcgtggtgatgtggagtattgccaacgaaccggatacccgtccgcaaggtgcacgggaatatttcgcgccactggcggaagcaacgcgtaaactcgacccgacgcgtccgatcacctgcgtcaatgtaatgttctgcgacgctcacaccgataccatcagcgatctctttgatgtgctgtgcctgaaccgttattacggatggtatgtccaaagcggcgatttggaaacggcagagaaggtactggaaaaagaacttctggcctggcaggagaaactgcatcagccgattatcatcaccgaatacggcgtggatacgttagccgggctgcactcaatgtacaccgacatgtggagtgaagagtatcagtgtgcatggctggatatgtatcaccgcgtctttgatcgcgtcagcgccgtcgtcggtgaacaggtatggaatttcgccgattttgcgacctcgcaaggcatattgcgcgttggcggtaacaagaaagggatcttcactcgcgaccgcaaaccgaagtcggcggcttttctgctgcaaaaacgctggactggcatgaacttcggtgaaaaaccgcagcagggaggcaaacaatga

SEQ ID NO: 43 - DNA, 928 bp, Artificial
  Synthetic EXP, EXP-At.GSP442+L-I-At.Cyco.
tgttaatgttatccgaactagtcataattacaaccgacaaaataaggttattttgtgtgttatagaattttttggacagtttttgttttggttttcgattgtagtaaaaatagatttatgtaataagatttacttttcttgttgaaacaaaataatcttagaattaactcaacttttatgttagaacaaatgataaaaaaatttccccttttctatgcgattattttcaatcagagagaaatacatataatatatataattcaaattaatctgccaaattaataaatttggattaaaatttataaatgaaacaatggtgtaaggcaattaaaaacacaacactaaaaatatgagaacattttatctgggcattaagagtttgggctttagatctaaaataaaggccggcccaacgagaatattaaaccctaattgacctagttccctatatatataaaccctatatttctctcgtcactcctcaactctcagctaaaccacggaccgcagtgagtcacataaccctcttggaaagagtctcaacacttgcagagaaaaagaacaaggaagatcccggaaacaggtaatttctctcctctctatttttaccattttccattgacgacgatctaggttttctgatttgattttggagaacgcctcgatgagtttatagattcgtagattggttttgagattcagtataatttcacccggattccaatttttgaaccgatacctaattttgaattgatttggtagatcgattggtcaaatttgaaattgatttttctccataatatctgaagcgtcttattggatcaaatctacaacatttctctgttgaaaggatcgattttttttttcttggaacatgataacttttgattattcatcaaagttttgttctttttaatatttcacaggt

SEQ ID NO: 44 - DNA, 300 bp, Artificial
  Synthetic 3' UTR, T-Zm.GST7.nno:2.
atgtctgctgcggcggccttcacagtttgtttatttcctactgtttgctgcggcgattgttgttgttttctgttttataaataataaaggaggaggagatttgttttggtttgtgtttgtttccatccttgctgctccatcacactatctgtaatttgtaaacagcgacaataaataaattaataaatttggtttctcatacctatatgtgtctgtttggaggcttgtttgtttgagacatctgtctggttgtttttttgctgccagccggtagtataaattttgtttttggacgacgaa

SEQ ID NO: 45 - DNA, 855 bp, Artificial
  Synthetic EXP, EXP-At.GSP576.nno+At.Cyco:1.
aattaaattcaacacgtttgttatatattttttattgaaattattcttcattcgtcttttaatggataaaaaggtataatcaagtatattttatacacatctttctatttgtgtgtaccaaatgttaaaatggccaattttgaccaaaaaaccgcataattttcttaatttcttaaatatgattaattcatcaataacttggaatttcacaatacacaaaagtgggtgtagttaccgttattatatttatacacaacaactcatctcctcatagaaagaaaagaaaaataaaataagaaatcaaaaaacgacaagataaccaatctccacatcatccacgtggcgtaaggataaggtcacaaccaccactcagccacgtggcagaatcttatccaatcactctcaccacacaaaccttatccacttctatatataatctcttcttctcattatcactcaccacacatccttgcaaaagtaaagagaaaaaacaaacaagacggaccgcaggtaatttctctcctctctatttttaccattttccattgacgacgatctaggttttctgatttgattttggagaacgcctcgatgagtttatagattcgtagattggttttgagattcagtataatttcacccggattccaatttttgaaccgatacctaattttgaattgatttggtagatcgattggtcaaatttgaaattgatttttctccataatatctgaagcgtcttattggatcaaatctacaacatttctctgttgaaaggatcgattttttttttcttggaacatgataacttttgattattcatcaaagttttgttctttttaatatttcacaggt

SEQ ID NO: 46 - DNA, 835 bp, Cauliflower mosaic virus
  misc_feature (1)..(835): DNA sequence of the EXP, EXP-CaMV.35S comprising the 35S promoter and leader derived from the Cauliflower mosaic virus.
agattagccttttcaatttcagaaagaatgctaacccacagatggttagagaggcttacgcagcaggtctcatcaagacgatctacccgagcaataatctccaggaaatcaaataccttcccaagaaggttaaagatgcagtcaaaagattcaggactaactgcatcaagaacacagagaaagatatatttctcaagatcagaagtactattccagtatggacgattcaaggcttgcttcacaaaccaaggcaagtaatagagattggagtctctaaaaaggtagttcccactgaatcaaaggccatggagtcaaagattcaaatagaggacctaacagaactcgccgtaaagactggcgaacagttcatacagagtctcttacgactcaatgacaagaagaaaatcttcgtcaacatggtggagcacgacacacttgtctactccaaaaatatcaaagatacagtctcagaagaccaaagggcaattgagacttttcaacaaagggtaatatccggaaacctcctcggattccattgcccagctatctgtcactttattgtgaagatagtggaaaaggaaggtggctcctacaaatgccatcattgcgataaaggaaaggccatcgttgaagatgcctctgccgacagtggtcccaaagatggacccccacccacgaggagcatcgtggaaaaagaagacgttccaaccacgtcttcaaagcaagtggattgatgtgatatctccactgacgtaagggatgacgcacaatcccactatccttcgcaagacccttcctctatataaggaagttcatttcatttggagaggacacg

SEQ ID NO: 47 - DNA, 804 bp, Zea mays
  misc_feature (1)..(804): DNA sequence of the intron, I-Zm.DnaK:1, derived from the heat shock protein 70 (Hsp70) gene (DnaK) from corn.
accgtcttcggtacgcgctcactccgccctctgcctttgttactgccacgtttctctgaatgctctcttgtgtggtgattgctgagagtggtttagctggatctagaattacactctgaaatcgtgttctgcctgtgctgattacttgccgtcctttgtagcagcaaaatatagggacatggtagtacgaaacgaagatagaacctacacagcaatacgagaaatgtgtaatttggtgcttagcggtatttatttaagcacatgttggtgttatagggcacttggattcagaagtttgctgttaatttaggcacaggcttcatactacatgggtcaatagtatagggattcatattataggcgatactataataatttgttcgtctgcagagcttattatttgccaaaattagatattcctattctgtttttgtttgtgtgctgttaaattgttaacgcctgaaggaataaatataaatgacgaaattttgatgtttatctctgctcctttattgtgaccataagtcaagatcagatgcacttgttttaaatattgttgtctgaagaaataagtactgacagtattttgatgcattgatctgcttgtttgttgtaacaaaatttaaaaataaagagtttcctttttgttgctctccttacctcctgatggtatctagtatctaccaactgacactatattgcttctctttacatacgtatcttgctcgatgccttctccctagtgttgaccagtgttactcacatagtctttgctcatttcattgtaatgcagataccaagcgg

SEQ ID NO: 48 - DNA, 300 bp, Orzya sativa
  misc_feature (1)..(300): DNA sequence of the 3' UTR, T-Os.LTP:1, derived from the Lipid Transfer Protein-like gene (LTP) from rice .
attaatcgatcctccgatcccttaattaccataccattacaccatgcatcaatatccatatatatataaaccctttcgcacgtacttatactatgttttgtcatacatatatatgtgtcgaacgatcgatctatcactgatatgatatgattgatccatcagcctgatctctgtatcttgttatttgtataccgtcaaataaaagtttcttccacttgtgttaataattagctactctcatctcatgaaccctatatataactagtttaatttgctgtcaattgaacatgatgatcgatg

SEQ ID NO: 49 - DNA, 516 bp, Artificial
  Coding sequence for an engineered luciferase flourescent protein.
atggtcttcacactcgaagatttcgttggggactggcgacagacagccggctacaacctggaccaagtccttgaacagggaggtgtgtccagtttgtttcagaatctcggggtgtccgtaactccgatccaaaggattgtcctgagcggtgaaaatgggctgaagatcgacatccatgtcatcatcccgtatgaaggtctgagcggcgaccaaatgggccagatcgaaaaaatttttaaggtggtgtaccctgtggatgatcatcactttaaggtgatcctgcactatggcacactggtaatcgacggggttacgccgaacatgatcgactatttcggacggccgtatgaaggcatcgccgtgttcgacggcaaaaagatcactgtaacagggaccctgtggaacggcaacaaaattatcgacgagcgcctgatcaaccccgacggctccctgctgttccgagtaaccatcaacggagtgaccggctggcggctgtgcgaacgcattctggcgtaa

SEQ ID NO: 50 - DNA, 1848 bp, Artificial
  DNA sequence of the EXP, EXP-At.Bglu21+At.Cyco:2 comprising the promoter and leader of a beta-glucuronidase 21 gene from Arabidopsis thaliana, operably linked 5' to the intron, I-At.Cyco-1:1:1.
aaataaatttcttaaagtgtgtgttttaatctaaaacatcatataatttgaaatagaggaaatatcatctaataaagtaatggtatatttgtatagttaatgatttgtctttttattcgcgcaaaatgtgtcaattataaaatataaagaggatataatttagtttagagttttagacacgaggactatatattggaaaacaaaaaagtaatgtaaaccatatagatcatggaatgagtcatcctattaaacagttgtattatatatttatattttagtcactaacacattaataacttaacgtccataacaaaataagatccaaaactcgatctagatctatacgaggcactaaatgatccattgacttagggccggccgattggttcgaggactcctcatgctgtaaactttttttttggacatacatgatatatttttaagtcacgtttttatattatatgttccacgcccaatataatatgttccaaactaggaaaaataagtaagaattagtcaatgatcgagataatgcaatgaatcatcctatttattaaatagatttactaaactatatataatacaatgatcgagatcgtgccatgaagcatcctatatactataaaaatagtcttactaaatacatactcatatagtttagtcattcattagtccaaacattaaatgagagatcctttacttgctacctgaattttttcagaataaggtataactttttttcgaattagaaactgatttatgaaagattaagagtaatgttcgttaaacaagttaaaaaatatgtttttacaattaagttttgaaaaataataaagtctccaattatttgagtatcaaaaataggcttgttattatttagggttttcgttggtttaaatgcaacggggtgtggttgtcattgtggaagttaatggaagtaattggttgaggttttaaacgttatcggacattttaaatgactggtttacagttaaaaatatgtgtatttacggcaattttatgattggcttagcagtagatgcgacagtggtttaaaccaaaaattaccaaataaataatatacaattattaaattatataaaacaccaatattatatatttatatatatatgaacatagttaattatcgaaaccatagacaaagtacataagagttattccgaaaaaggtttattatgaaacacaaataatcatattgggagattatgatatccaaaatggactaatcaaataattaaatccaaaatggatgaagaacttatattagttccacgcacaatataatatgttccaaactaagtaagaacacaacggtcgaggtcatgcaatgaatcatcctatatataaaatagttttactaaacaattatattttagtcactcgttaacaaacaatcaaaatcgctatataaagaactccgattggatgtaaacaaatcatcataaacttgttctcttccagaagaaactaaaaacaaaacaggtaatttctctcctctctatttttaccattttccattgacgacgatctaggttttctgatttgattttggagaacgcctcgatgagtttatagattcgtagattggttttgagattcagtataatttcacccggattccaatttttgaaccgatacctaattttgaattgatttggtagatcgattggtcaaatttgaaattgatttttctccataatatctgaagcgtcttattggatcaaatctacaacatttctctgttgaaaggatcgattttttttttcttggaacatgataacttttgattattcatcaaagttttgttctttttaatatttcacaggt

SEQ ID NO: 51 - DNA, 712 bp, Artificial
  DNA sequence of the EXP, EXP-CaMV.35S-enh+Ph.DnaK:1:3 comprising an enhanced Cauliflower mosaic virus 35S promoter, operably linked 5' to the leader of the heat shock protein 70 (HSP70) gene from Petunia.
ggtccgatgtgagacttttcaacaaagggtaatatccggaaacctcctcggattccattgcccagctatctgtcactttattgtgaagatagtggaaaaggaaggtggctcctacaaatgccatcattgcgataaaggaaaggccatcgttgaagatgcctctgccgacagtggtcccaaagatggacccccacccacgaggagcatcgtggaaaaagaagacgttccaaccacgtcttcaaagcaagtggattgatgtgatggtccgattgagacttttcaacaaagggtaatatccggaaacctcctcggattccattgcccagctatctgtcactttattgtgaagatagtggaaaaggaaggtggctcctacaaatgccatcattgcgataaaggaaaggccatcgttgaagatgcctctgccgacagtggtcccaaagatggacccccacccacgaggagcatcgtggaaaaagaagacgttccaaccacgtcttcaaagcaagtggattgatgtgatatctccactgacgtaagggatgacgcacaatcccactatccttcgcaagacccttcctctatataaggaagttcatttcatttggagaggacactctagacagaaaaatttgctacattgtttcacaaacttcaaatattattcatttatttgtcagctttcaaactctttgtttcttgtttgttgatt

SEQ ID NO: 52 - DNA, 841 bp, Glycine max
  misc_feature (1)..(841): DNA sequence of the EXP, EXP-Gm.Sphas1:1:1 comprising the promoter and leader of the 7S alpha prime gene of soybean.
ggcaaaaacatttaatacgtattatttaagaaaaaaatatgtaataatatatttatattttaatatctattcttatgtattttttaaaaatctattatatattgatcaactaaaatatttttatatctacacttattttgcatttttatcaattttcttgcgttttttggcatatttaataatgactattctttaataatcaatcattattcttacatggtacatattgttggaaccatatgaagtgtccattgcatttgactatgtggatagtgttttgatccaggcctccatttgccgcttattaattaatttggtaacagtccgtactaatcagttacttatccttcctccatcataattaatcttggtagtctcgaatgccacaacactgactagtctcttggatcataagaaaaagccaaggaacaaaagaagacaaaacacaatgagagtatcctttgcatagcaatgtctaagttcataaaattcaaacaaaaacgcaatcacacacagtggacatcacttatccactagctgatcaggatcgccgcgtcaagaaaaaaaaactggaccccaaaagccatgcacaacaacacgtactcacaaaggtgtcaatcgagcagcccaaaacattcaccaactcaacccatcatgagcccacacatttgttgtttctaacccaacctcaaactcgtattctcttccgccacctcatttttgtttatttcaacacccgtcaaactgcatgccaccccgtggccaaatgtccatgcatgttaacaagacctatgactataaatatctgcaatctcggcccaggttttcatcatcaagaacc

SEQ ID NO: 53 - DNA, 1446 bp, Artificial
  DNA sequence of the EXP, EXP-CaMV.35S-enh+Zm.DnaK:1:1 comprising an enhanced Cauliflower mosaic virus 35S promoter, operably linked 5' to the intron, I-Zm.DnaK:1.
ggtccgattgagacttttcaacaaagggtaatatccggaaacctcctcggattccattgcccagctatctgtcactttattgtgaagatagtggaaaaggaaggtggctcctacaaatgccatcattgcgataaaggaaaggccatcgttgaagatgcctctgccgacagtggtcccaaagatggacccccacccacgaggagcatcgtggaaaaagaagacgttccaaccacgtcttcaaagcaagtggattgatgtgatggtccgattgagacttttcaacaaagggtaatatccggaaacctcctcggattccattgcccagctatctgtcactttattgtgaagatagtggaaaaggaaggtggctcctacaaatgccatcattgcgataaaggaaaggccatcgttgaagatgcctctgccgacagtggtcccaaagatggacccccacccacgaggagcatcgtggaaaaagaagacgttccaaccacgtcttcaaagcaagtggattgatgtgatatctccactgacgtaagggatgacgcacaatcccactatccttcgcaagacccttcctctatataaggaagttcatttcatttggagaggacacgctgacaagctgactctagcagatctaccgtcttcggtacgcgctcactccgccctctgcctttgttactgccacgtttctctgaatgctctcttgtgtggtgattgctgagagtggtttagctggatctagaattacactctgaaatcgtgttctgcctgtgctgattacttgccgtcctttgtagcagcaaaatatagggacatggtagtacgaaacgaagatagaacctacacagcaatacgagaaatgtgtaatttggtgcttagcggtatttatttaagcacatgttggtgttatagggcacttggattcagaagtttgctgttaatttaggcacaggcttcatactacatgggtcaatagtatagggattcatattataggcgatactataataatttgttcgtctgcagagcttattatttgccaaaattagatattcctattctgtttttgtttgtgtgctgttaaattgttaacgcctgaaggaataaatataaatgacgaaattttgatgtttatctctgctcctttattgtgaccataagtcaagatcagatgcacttgttttaaatattgttgtctgaagaaataagtactgacagtattttgatgcattgatctgcttgtttgttgtaacaaaatttaaaaataaagagtttcctttttgttgctctccttacctcctgatggtatctagtatctaccaactgacactatattgcttctctttacatacgtatcttgctcgatgccttctccctagtgttgaccagtgttactcacatagtctttgctcatttcattgtaatgcagataccaagcgg

SEQ ID NO: 54 - DNA, 1653 bp, Photinus pyralis
  misc_feature (1)..(1653): DNA sequence encoding a luciferase protein derived from Firefly.
atggaagacgccaaaaacataaagaaaggcccggcgccattctatcctctagaggatggaaccgctggagagcaactgcataaggctatgaagagatacgccctggttcctggaacaattgcttttacagatgcacatatcgaggtgaacatcacgtacgcggaatacttcgaaatgtccgttcggttggcagaagctatgaaacgatatgggctgaatacaaatcacagaatcgtcgtatgcagtgaaaactctcttcaattctttatgccggtgttgggcgcgttatttatcggagttgcagttgcgcccgcgaacgacatttataatgaacgtgaattgctcaacagtatgaacatttcgcagcctaccgtagtgtttgtttccaaaaaggggttgcaaaaaattttgaacgtgcaaaaaaaattaccaataatccagaaaattattatcatggattctaaaacggattaccagggatttcagtcgatgtacacgttcgtcacatctcatctacctcccggttttaatgaatacgattttgtaccagagtcctttgatcgtgacaaaacaattgcactgataatgaattcctctggatctactgggttacctaagggtgtggcccttccgcatagaactgcctgcgtcagattctcgcatgccagagatcctatttttggcaatcaaatcattccggatactgcgattttaagtgttgttccattccatcacggttttggaatgtttactacactcggatatttgatatgtggatttcgagtcgtcttaatgtatagatttgaagaagagctgtttttacgatcccttcaggattacaaaattcaaagtgcgttgctagtaccaaccctattttcattcttcgccaaaagcactctgattgacaaatacgatttatctaatttacacgaaattgcttctgggggcgcacctctttcgaaagaagtcggggaagcggttgcaaaacgcttccatcttccagggatacgacaaggatatgggctcactgagactacatcagctattctgattacacccgagggggatgataaaccgggcgcggtcggtaaagttgttccattttttgaagcgaaggttgtggatctggataccgggaaaacgctgggcgttaatcagagaggcgaattatgtgtcagaggacctatgattatgtccggttatgtaaacaatccggaagcgaccaacgccttgattgacaaggatggatggctacattctggagacatagcttactgggacgaagacgaacacttcttcatagttgaccgcttgaagtctttaattaaatacaaaggatatcaggtggcccccgctgaattggaatcgatattgttacaacaccccaacatcttcgacgcgggcgtggcaggtcttcccgacgatgacgccggtgaacttcccgccgccgttgttgttttggagcacggaaagacgatgacggaaaaagagatcgtggattacgtcgccagtcaagtaacaaccgcgaaaaagttgcgcggaggagttgtgtttgtggacgaagtaccgaaaggtcttaccggaaaactcgacgcaagaaaaatcagagagatcctcataaaggccaagaagggcggaaagtccaaattgtaa

SEQ ID NO: 55 - DNA, 253 bp, Agrobacterium tumefaciens
  misc_feature (1)..(253): DNA sequence of the 3' UTR, T-AGRtu.nos-1:1:13 derived from the Agrobacterium tumefaciens nopaline synthase gene.
gatcgttcaaacatttggcaataaagtttcttaagattgaatcctgttgccggtcttgcgatgattatcatataatttctgttgaattacgttaagcatgtaataattaacatgtaatgcatgacgttatttatgagatgggtttttatgattagagtcccgcaattatacatttaatacgcgatagaaaacaaaatatagcgcgcaaactaggataaattatcgcgcgcggtgtcatctatgttactagatc

SEQ ID NO: 56 - DNA, 675 bp, Artificial
  DNA sequence of the EXP,  EXP-CaMV.35S-enh-Lhcb1 comprising an enhanced Cauliflower mosaic virus 35S promoter, operably linked 5' to the leader of a chlorophyll a/b-binding gene of the light-harvesting complex of wheat.
ggtccgatgtgagacttttcaacaaagggtaatatccggaaacctcctcggattccattgcccagctatctgtcactttattgtgaagatagtggaaaaggaaggtggctcctacaaatgccatcattgcgataaaggaaaggccatcgttgaagatgcctctgccgacagtggtcccaaagatggacccccacccacgaggagcatcgtggaaaaagaagacgttccaaccacgtcttcaaagcaagtggattgatgtgatggtccgatgtgagacttttcaacaaagggtaatatccggaaacctcctcggattccattgcccagctatctgtcactttattgtgaagatagtggaaaaggaaggtggctcctacaaatgccatcattgcgataaaggaaaggccatcgttgaagatgcctctgccgacagtggtcccaaagatggacccccacccacgaggagcatcgtggaaaaagaagacgttccaaccacgtcttcaaagcaagtggattgatgtgatatctccactgacgtaagggatgacgcacaatcccactatccttcgcaagacccttcctctatataaggaagttcatttcatttggagaggaaccatcttccacacactcaagccacactattggagaacacacagggacaacacaccataa

SEQ ID NO: 57 - DNA, 936 bp, Renilla reniformis
  misc_feature (1)..(936): DNA sequence encoding a luciferase protein derived from Sea Pansey.
atggcttccaaggtgtacgaccccgagcaacgcaaacgcatgatcactgggcctcagtggtgggctcgctgcaagcaaatgaacgtgctggactccttcatcaactactatgattccgagaagcacgccgagaacgccgtgatttttctgcatggtaacgctgcctccagctacctgtggaggcacgtcgtgcctcacatcgagcccgtggctagatgcatcatccctgatctgatcggaatgggtaagtccggcaagagcgggaatggctcatatcgcctcctggatcactacaagtacctcaccgcttggttcgagctgctgaaccttccaaagaaaatcatctttgtgggccacgactggggggcttgtctggcctttcactactcctacgagcaccaagacaagatcaaggccatcgtccatgctgagagtgtcgtggacgtgatcgagtcctgggacgagtggcctgacatcgaggaggatatcgccctgatcaagagcgaagagggcgagaaaatggtgcttgagaataacttcttcgtcgagaccatgctcccaagcaagatcatgcggaaactggagcctgaggagttcgctgcctacctggagccattcaaggagaagggcgaggttagacggcctaccctctcctggcctcgcgagatccctctcgttaagggaggcaagcccgacgtcgtccagattgtccgcaactacaacgcctaccttcgggccagcgacgatctgcctaagatgttcatcgagtccgaccctgggttcttttccaacgctattgtcgagggagctaagaagttccctaacaccgagttcgtgaaggtgaagggcctccacttcagccaggaggacgctccagatgaaatgggtaagtacatcaagagcttcgtggagcgcgtgctgaagaacgagcagtaa